European Patent Specification EP 3 433 598 B1, published September 18, 2024. Title: BILLES SOLUBLES POUR LA PRÉPARATION DE SOLUTIONS. Applicant: ANAQUANT. The sequence listing filed with the application follows.

SEQUENCE LISTING (160 sequences)

SEQ ID NO: 1 - protein, 9 aa, Séquence artificielle
  Peptide
EGVLYVGSK

SEQ ID NO: 2 - protein, 9 aa, Séquence artificielle
  peptide
EGVVAAAEK

SEQ ID NO: 3 - protein, 13 aa, Séquence artificielle
  peptide
EGVVHGVTTVAEK

SEQ ID NO: 4 - protein, 20 aa, Séquence artificielle
  peptide
EQVTNVGGAVVTGVTAVAQK

SEQ ID NO: 5 - protein, 9 aa, Séquence artificielle
  peptide
QGVAEAAGK

SEQ ID NO: 6 - protein, 16 aa, Séquence artificielle
  peptide
TVEGAGNIAAATGFVK

SEQ ID NO: 7 - protein, 26 aa, Séquence artificielle
  peptide
AEEAGIGDTPNQEDQAAGHVTPHQAR

SEQ ID NO: 8 - protein, 24 aa, Séquence artificielle
  peptide
AEEAGIGDTPNQEDQAAGHVTQAR

SEQ ID NO: 9 - protein, 26 aa, Séquence artificielle
  peptide
AEEAGIGDTPSLEDEAAGHVTPHQAR

SEQ ID NO: 10 - protein, 24 aa, Séquence artificielle
  peptide
AEEAGIGDTPSLEDEAAGHVTQAR

SEQ ID NO: 11 - protein, 22 aa, Séquence artificielle
  peptide
CCAMGSLGNIHHKPGGGQVEVK

SEQ ID NO: 12 - protein, 8 aa, Séquence artificielle
  peptide
DRTGNDEK

SEQ ID NO: 13 - protein, 25 aa, Séquence artificielle
  peptide
ESPHPLQTPTEDGSEEPGSETSDAK

SEQ ID NO: 14 - protein, 25 aa, Séquence artificielle
  peptide
ESPHPPQPPADDGAEEPGSETSDAK

SEQ ID NO: 15 - protein, 23 aa, Séquence artificielle
  peptide
ESPLQTPTEDGSEEPGSETSDAK

SEQ ID NO: 16 - protein, 23 aa, Séquence artificielle
  peptide
ESPPQPPADDGAEEPGSETSDAK

SEQ ID NO: 17 - protein, 8 aa, Séquence artificielle
  peptide
GAAPPGQK

SEQ ID NO: 18 - protein, 8 aa, Séquence artificielle
  peptide
GAASPAQK

SEQ ID NO: 19 - protein, 32 aa, Séquence artificielle
  peptide
HLSNVSSTGSIDMVDSPQLATLADEVSASLAK

SEQ ID NO: 20 - protein, 19 aa, Séquence artificielle
  peptide
HVLGGGSVQIVYKPVDLSK

SEQ ID NO: 21 - protein, 19 aa, Séquence artificielle
  peptide
HVPGGGSVQIVYKPVDLSK

SEQ ID NO: 22 - protein, 13 aa, Séquence artificielle
  peptide
IATPRGAAPPGQK

SEQ ID NO: 23 - protein, 12 aa, Séquence artificielle
  peptide
TFDPYYAVALVK

SEQ ID NO: 24 - protein, 12 aa, Séquence artificielle
  peptide
FTDPVNIISVYK

SEQ ID NO: 25 - protein, 17 aa, Séquence artificielle
  peptide
LGDPLGADVAQVTGALR

SEQ ID NO: 26 - protein, 12 aa, Séquence artificielle
  peptide
GIDPEAVLADLR

SEQ ID NO: 27 - protein, 15 aa, Séquence artificielle
  peptide
YDPLVVFSHGLGAFR

SEQ ID NO: 28 - protein, 12 aa, Séquence artificielle
  peptide
QDPNEILIFWSK

SEQ ID NO: 29 - protein, 22 aa, Séquence artificielle
  peptide
EQDPVTNVGGAVVTGVTAVAQK

SEQ ID NO: 30 - protein, 12 aa, Séquence artificielle
  peptide
IDPGSSDGSSSR

SEQ ID NO: 31 - protein, 11 aa, Séquence artificielle
  peptide
EGDPVVAAAEK

SEQ ID NO: 32 - protein, 11 aa, Séquence artificielle
  peptide
EADPNYIGSDK

SEQ ID NO: 33 - protein, 13 aa, Séquence artificielle
  peptide
SQDPTVLQNTGGR

SEQ ID NO: 34 - protein, 11 aa, Séquence artificielle
  peptide
SGDPGVCLNCR

SEQ ID NO: 35 - protein, 11 aa, Séquence artificielle
  peptide
ATDPFNPAQDK

SEQ ID NO: 36 - protein, 11 aa, Séquence artificielle
  peptide
ANDPIGATLNR

SEQ ID NO: 37 - protein, 11 aa, Séquence artificielle
  peptide
LYYDPSQDNDR

SEQ ID NO: 38 - protein, 9 aa, Séquence artificielle
  peptide
SDPIAPCIK

SEQ ID NO: 39 - protein, 11 aa, Séquence artificielle
  peptide
SLADPAVVTGK

SEQ ID NO: 40 - protein, 7 aa, Séquence artificielle
  peptide
TLDPFSR

SEQ ID NO: 41 - protein, 18 aa, Séquence artificielle
  peptide
LHDPTFGDENEDDSELAR

SEQ ID NO: 42 - protein, 10 aa, Séquence artificielle
  peptide
ASDPYLDCIK

SEQ ID NO: 43 - protein, 18 aa, Séquence artificielle
  peptide
IGDPSLDNITHVPGGGNK

SEQ ID NO: 44 - protein, 14 aa, Séquence artificielle
  peptide
ADPAATVVDVDEVR

SEQ ID NO: 45 - protein, 6 aa, Séquence artificielle
  peptide
VQIINK

SEQ ID NO: 46 - protein, 14 aa, Séquence artificielle
  peptide
VQIVYPHKPVDLSK

SEQ ID NO: 47 - protein, 15 aa, Séquence artificielle
  peptide
AVFVDLEPTVIDEVR

SEQ ID NO: 48 - protein, 18 aa, Séquence artificielle
  peptide
VGINYQPPTVVPGGDLAK

SEQ ID NO: 49 - protein, 18 aa, Séquence artificielle
  peptide
VAPEEHPVLLTEAPLNPK

SEQ ID NO: 50 - protein, 10 aa, Séquence artificielle
  peptide
DVNAAIAAIK

SEQ ID NO: 51 - protein, 9 aa, Séquence artificielle
  peptide
EIIDPVLDR

SEQ ID NO: 52 - protein, 11 aa, Séquence artificielle
  peptide
DSYVGDEAQSK

SEQ ID NO: 53 - protein, 11 aa, Séquence artificielle
  peptide
AVFPSIVGRPR

SEQ ID NO: 54 - protein, 9 aa, Séquence artificielle
  peptide
GIAPLQLGK

SEQ ID NO: 55 - protein, 16 aa, Séquence artificielle
  peptide
LHTFGDENEDDSELAR

SEQ ID NO: 56 - protein, 9 aa, Séquence artificielle
  peptide
SGGVCLNCR

SEQ ID NO: 57 - protein, 8 aa, Séquence artificielle
  peptide
SPIAPCIK

SEQ ID NO: 58 - protein, 8 aa, Séquence artificielle
  peptide
SSLVIQWR

SEQ ID NO: 59 - protein, 14 aa, Séquence artificielle
  peptide
FDPVHAALVWGPEK

SEQ ID NO: 60 - protein, 10 aa, Séquence artificielle
  peptide
SYDPYWIGIR

SEQ ID NO: 61 - protein, 13 aa, Séquence artificielle
  peptide
IATPRGAASPAQK

SEQ ID NO: 62 - protein, 18 aa, Séquence artificielle
  peptide
IGSPHLDNITHVPGGGNK

SEQ ID NO: 63 - protein, 10 aa, Séquence artificielle
  peptide
IGSPHTENLK

SEQ ID NO: 64 - protein, 16 aa, Séquence artificielle
  peptide
IGSLDNITHVPGGGNK

SEQ ID NO: 65 - protein, 8 aa, Séquence artificielle
  peptide
IGSTENLK

SEQ ID NO: 66 - protein, 11 aa, Séquence artificielle
  peptide
LDLSNVQSPHK

SEQ ID NO: 67 - protein, 9 aa, Séquence artificielle
  peptide
LDLSNVQSK

SEQ ID NO: 68 - protein, 12 aa, Séquence artificielle
  peptide
LQTAPVPMPDLK

SEQ ID NO: 69 - protein, 28 aa, Séquence artificielle
  peptide
QEFDTMEDHAGDYTLLQDQEGDMDHGLK

SEQ ID NO: 70 - protein, 19 aa, Séquence artificielle
  peptide
QEFEVMIEDHAGTYGLGDR

SEQ ID NO: 71 - protein, 18 aa, Séquence artificielle
  peptide
QEFEVMEDHAGTYGLGDR

SEQ ID NO: 72 - protein, 15 aa, Séquence artificielle
  peptide
SPHPVVSGDTSPHPR

SEQ ID NO: 73 - protein, 13 aa, Séquence artificielle
  peptide
SPHPVVSGDTSPR

SEQ ID NO: 74 - protein, 24 aa, Séquence artificielle
  peptide
SPHTPTPHAEDVTAPLVDEGAPGK

SEQ ID NO: 75 - protein, 20 aa, Séquence artificielle
  peptide
SPHTPTPHAEDVTAPLVDER

SEQ ID NO: 76 - protein, 22 aa, Séquence artificielle
  peptide
SPHTPTAEDVTAPLVDEGAPGK

SEQ ID NO: 77 - protein, 18 aa, Séquence artificielle
  peptide
SPHTPTAEDVTAPLVDER

SEQ ID NO: 78 - protein, 19 aa, Séquence artificielle
  peptide
SGYSSPGSPHPGTPHPGSR

SEQ ID NO: 79 - protein, 17 aa, Séquence artificielle
  peptide
SGYSSPGSPHPGTPGSR

SEQ ID NO: 80 - protein, 17 aa, Séquence artificielle
  peptide
SGYSSPGSPGTPHPGSR

SEQ ID NO: 81 - protein, 15 aa, Séquence artificielle
  peptide
SGYSSPGSPGTPGSR

SEQ ID NO: 82 - protein, 13 aa, Séquence artificielle
  peptide
SPVVSGDTSPHPR

SEQ ID NO: 83 - protein, 11 aa, Séquence artificielle
  peptide
SPVVSGDTSPR

SEQ ID NO: 84 - protein, 22 aa, Séquence artificielle
  peptide
STPTPHAEDVTAPLVDEGAPGK

SEQ ID NO: 85 - protein, 18 aa, Séquence artificielle
  peptide
STPTPHAEDVTAPLVDER

SEQ ID NO: 86 - protein, 20 aa, Séquence artificielle
  peptide
STPTAEDVTAPLVDEGAPGK

SEQ ID NO: 87 - protein, 16 aa, Séquence artificielle
  peptide
STPTAEDVTAPLVDER

SEQ ID NO: 88 - protein, 10 aa, Séquence artificielle
  peptide
VDPSVYPLDR

SEQ ID NO: 89 - protein, 13 aa, Séquence artificielle
  peptide
EGDPYYGYTGAFR

SEQ ID NO: 90 - protein, 10 aa, Séquence artificielle
  peptide
DSDPAYGFFK

SEQ ID NO: 91 - protein, 9 aa, Séquence artificielle
  peptide
VEDPSWILR

SEQ ID NO: 92 - protein, 10 aa, Séquence artificielle
  peptide
SSDPLVIQWR

SEQ ID NO: 93 - protein, 12 aa, Séquence artificielle
  peptide
CIPDFVNAAFGK

SEQ ID NO: 94 - protein, 38 aa, Séquence artificielle
  peptide
TCTTPAQGNSMFPSCCCTKPTDGNCTCIPIPSSWAFAK

SEQ ID NO: 95 - protein, 22 aa, Séquence artificielle
  peptide
TCTTPAQGNSMFPSCCCTKPTD

SEQ ID NO: 96 - protein, 16 aa, Séquence artificielle
  peptide
GNCTCIPIPSSWAFAK

SEQ ID NO: 97 - protein, 19 aa, Séquence artificielle
  peptide
KTCTTPAQGNSMFPSCCCT

SEQ ID NO: 98 - protein, 19 aa, Séquence artificielle
  peptide
KPTDGNCTCIPIPSSWAFA

SEQ ID NO: 99 - protein, 19 aa, Séquence artificielle
  peptide
TCTTPAQGNSMFPSCCCTK

SEQ ID NO: 100 - protein, 19 aa, Séquence artificielle
  peptide
PTDGNCTCIPIPSSWAFAK

SEQ ID NO: 101 - protein, 9 aa, Séquence artificielle
  peptide
LGPLVEQGR

SEQ ID NO: 102 - protein, 18 aa, Séquence artificielle
  peptide
LGATQSNEITIPVTFESR

SEQ ID NO: 103 - protein, 19 aa, Séquence artificielle
  peptide
NGVPQEESLEDSDVDADFK

SEQ ID NO: 104 - protein, 14 aa, Séquence artificielle
  peptide
LGASVPGSQTVVVK

SEQ ID NO: 105 - protein, 9 aa, Séquence artificielle
  peptide
NGISQVLEK

SEQ ID NO: 106 - protein, 8 aa, Séquence artificielle
  peptide
NGFSIQVR

SEQ ID NO: 107 - protein, 7 aa, Séquence artificielle
  peptide
DGVTLQK

SEQ ID NO: 108 - protein, 13 aa, Séquence artificielle
  peptide
SGIPDNAFQSFGR

SEQ ID NO: 109 - protein, 17 aa, Séquence artificielle
  peptide
LGLIFDTSNLQSGVPSR

SEQ ID NO: 110 - protein, 8 aa, Séquence artificielle
  peptide
LGPQTLSR

SEQ ID NO: 111 - protein, 14 aa, Séquence artificielle
  peptide
TPHPPGSPHGEPPK

SEQ ID NO: 112 - protein, 12 aa, Séquence artificielle
  peptide
TPHPPGSGEPPK

SEQ ID NO: 113 - protein, 9 aa, Séquence artificielle
  peptide
EGQLTPLIK

SEQ ID NO: 114 - protein, 12 aa, Séquence artificielle
  peptide
EGFDDLPLAEQR

SEQ ID NO: 115 - protein, 15 aa, Séquence artificielle
  peptide
TGQSSLVPALTDFVR

SEQ ID NO: 116 - protein, 9 aa, Séquence artificielle
  peptide
GIAPLQLGK

SEQ ID NO: 117 - protein, 14 aa, Séquence artificielle
  peptide
IAKPNVSASTQASR

SEQ ID NO: 118 - protein, 10 aa, Séquence artificielle
  peptide
TLDFHDSNVK

SEQ ID NO: 119 - protein, 8 aa, Séquence artificielle
  peptide
VLPEDGPR

SEQ ID NO: 120 - protein, 8 aa, Séquence artificielle
  peptide
YLGADYIK

SEQ ID NO: 121 - protein, 14 aa, Séquence artificielle
  peptide
TPHPPSSPHGEPPK

SEQ ID NO: 122 - protein, 12 aa, Séquence artificielle
  peptide
TPHPPSSGEPPK

SEQ ID NO: 123 - protein, 14 aa, Séquence artificielle
  peptide
TPHPSPHLPTPPTR

SEQ ID NO: 124 - protein, 12 aa, Séquence artificielle
  peptide
TDHGAEIVYPHK

SEQ ID NO: 125 - protein, 10 aa, Séquence artificielle
  peptide
TDHGAEIVYK

SEQ ID NO: 126 - protein, 12 aa, Séquence artificielle
  peptide
TPPGSPHGEPPK

SEQ ID NO: 127 - protein, 10 aa, Séquence artificielle
  peptide
TPPGSGEPPK

SEQ ID NO: 128 - protein, 12 aa, Séquence artificielle
  peptide
TPPSSPHGEPPK

SEQ ID NO: 129 - protein, 10 aa, Séquence artificielle
  peptide
TPPSSGEPPK

SEQ ID NO: 130 - protein, 12 aa, Séquence artificielle
  peptide
TPSPHLPTPPTR

SEQ ID NO: 131 - protein, 10 aa, Séquence artificielle
  peptide
TPSLPTPPTR

SEQ ID NO: 132 - protein, 11 aa, Séquence artificielle
  peptide
VAVVRTPHPPK

SEQ ID NO: 133 - protein, 9 aa, Séquence artificielle
  peptide
VAVVRTPPK

SEQ ID NO: 134 - protein, 12 aa, Séquence artificielle
  peptide
VQIVYKPVDLSK

SEQ ID NO: 135 - protein, 34 aa, Séquence artificielle
  peptide
HLSNVSSPHTGSIDMVDSPQLATLADEVSASLAK

SEQ ID NO: 136 - protein, 21 aa, Séquence artificielle
  peptide
HVPGGGSVQIVYPHKPVDLSK

SEQ ID NO: 137 - protein, 19 aa, Séquence artificielle
  peptide
HVSGGGSVQIVYKPVDLSK

SEQ ID NO: 138 - protein, 17 aa, Séquence artificielle
  peptide
SGYSSPHPGSPGTPGSR

SEQ ID NO: 139 - protein, 12 aa, Séquence artificielle
  peptide
TPHPSLPTPPTR

SEQ ID NO: 140 - protein, 12 aa, Séquence artificielle
  peptide
TPSLPTPHPPTR

SEQ ID NO: 141 - protein, 16 aa, Séquence artificielle
  peptide
GGFPEFVNELHNNGQK

SEQ ID NO: 142 - protein, 11 aa, Séquence artificielle
  peptide
EGAQLPVIENK

SEQ ID NO: 143 - protein, 11 aa, Séquence artificielle
  peptide
AGIPNNQVLGK

SEQ ID NO: 144 - protein, 8 aa, Séquence artificielle
  peptide
ALVQIVGK

SEQ ID NO: 145 - protein, 9 aa, Séquence artificielle
  peptide
GHSGLQPGR

SEQ ID NO: 146 - protein, 15 aa, Séquence artificielle
  peptide
ASTPGAAAQIQEVGK

SEQ ID NO: 147 - protein, 8 aa, Séquence artificielle
  peptide
VVNPTQGK

SEQ ID NO: 148 - protein, 11 aa, Séquence artificielle
  peptide
IPLENLQIIGR

SEQ ID NO: 149 - protein, 9 aa, Séquence artificielle
  peptide
NLAVQAQGK

SEQ ID NO: 150 - protein, 10 aa, Séquence artificielle
  peptide
VLDALQAIGK

SEQ ID NO: 151 - protein, 16 aa, Séquence artificielle
  peptide
VTEPISAESGEQVEGR

SEQ ID NO: 152 - protein, 15 aa, Séquence artificielle
  peptide
ISPNTSQQNFVTQGR

SEQ ID NO: 153 - protein, 17 aa, Séquence artificielle
  peptide
FQAFANGSLLIPDFGGK

SEQ ID NO: 154 - protein, 13 aa, Séquence artificielle
  peptide
EPISVSSEQVLGK

SEQ ID NO: 155 - protein, 15 aa, Séquence artificielle
  peptide
AVFQANQENLPILGK

SEQ ID NO: 156 - protein, 12 aa, Séquence artificielle
  peptide
VQPVSEILQLGK

SEQ ID NO: 157 - protein, 10 aa, Séquence artificielle
  peptide
ALDVIQAGGK

SEQ ID NO: 158 - protein, 12 aa, Séquence artificielle
  peptide
IIHESGAQILGR

SEQ ID NO: 159 - protein, 11 aa, Séquence artificielle
  peptide
EQLSSVSSFER

SEQ ID NO: 160 - protein, 7 aa, Séquence artificielle
  peptide
GDVAFVK